European Patent Application EP 4 269 684 A2, published November 1, 2023. Title: ALPHA-AMYLASE WITH ALTERED PROPERTIES. Applicant: Novozymes A/S. Application EP. The sequence listing filed with the application follows.

SEQUENCE LISTING (18 sequences)

SEQ ID NO: 1 - DNA, 1455 bp, Bacillus SP690
  source 1..1455: mol_type = genomic DNA
catcataatggaacaaatggtactatgatgcaatatttcgaatggtatttgccaaatgacgggaatcattggaacaggttgagggatgacgcagctaacttaaagagtaaagggataacagctgtatggatcccacctgcatggaaggggacttcccagaatgatgtaggttatggagcctatgatttatatgatcttggagagtttaaccagaaggggacggttcgtacaaaatatggaacacgcaaccagctacaggctgcggtgacctctttaaaaaataacggcattcaggtatatggtgatgtcgtcatgaatcataaaggtggagcagatggtacggaaattgtaaatgcggtagaagtgaatcggagcaaccgaaaccaggaaacctcaggagagtatgcaatagaagcgtggacaaagtttgattttcctggaagaggaaataaccattccagctttaagtggcgctggtatcattttgatgggacagattgggatcagtcacgccagcttcaaaacaaaatatataaattcaggggaacaggcaaggcctgggactgggaagtcgatacagagaatggcaactatgactatcttatgtatgcagacgtggatatggatcacccagaagtaatacatgaacttagaaactggggagtgtggtatacgaatacactgaaccttgatggatttagaatagatgcagtgaaacatataaaatatagctttacgagagattggcttacacatgtgcgtaacaccacaggtaaaccaatgtttgcagtggctgagttttggaaaaatgaccttggtgcaattgaaaactatttgaataaaacaagttggaatcactcggtgtttgatgttcctctccactataatttgtacaatgcatctaatagcggtggttattatgatatgagaaatattttaaatggttctgtggtgcaaaaacatccaacacatgccgttacttttgttgataaccatgattctcagcccggggaagcattggaatcctttgttcaacaatggtttaaaccacttgcatatgcattggttctgacaagggaacaaggttatccttccgtattttatggggattactacggtatcccaacccatggtgttccggctatgaaatctaaaatagaccctcttctgcaggcacgtcaaacttttgcctatggtacgcagcatgattactttgatcatcatgatattatcggttggacaagagagggaaatagctcccatccaaattcaggccttgccaccattatgtcagatggtccaggtggtaacaaatggatgtatgtggggaaaaataaagcgggacaagtttggagagatattaccggaaataggacaggcaccgtcacaattaatgcagacggatggggtaatttctctgttaatggagggtccgtttcggtttgggtgaagcaa

SEQ ID NO: 2 - protein, 485 aa, Bacillus SP690
HHNGTNGTMMQYFEWYLPNDGNHWNRLRDDAANLKSKGITAVWIPPAWKGTSQNDVGYGAYDLYDLGEFNQKGTVRTKYGTRNQLQAAVTSLKNNGIQVYGDVVMNHKGGADGTEIVNAVEVNRSNRNQETSGEYAIEAWTKFDFPGRGNNHSSFKWRWYHFDGTDWDQSRQLQNKIYKFRGTGKAWDWEVDTENGNYDYLMYADVDMDHPEVIHELRNWGVWYTNTLNLDGFRIDAVKHIKYSFTRDWLTHVRNTTGKPMFAVAEFWKNDLGAIENYLNKTSWNHSVFDVPLHYNLYNASNSGGYYDMRNILNGSVVQKHPTHAVTFVDNHDSQPGEALESFVQQWFKPLAYALVLTREQGYPSVFYGDYYGIPTHGVPAMKSKIDPLLQARQTFAYGTQHDYFDHHDIIGWTREGNSSHPNSGLATIMSDGPGGNKWMYVGKNKAGQVWRDITGNRTGTVTINADGWGNFSVNGGSVSVWVKQ

SEQ ID NO: 3 - DNA, 1455 bp, Bacillus SP722
  source 1..1455: mol_type = genomic DNA
  CDS 1..1455
catcataatgggacaaatgggacgatgatgcaatactttgaatggcacttgcctaatgatgggaatcactggaatagattaagagatgatgctagtaatctaagaaatagaggtataaccgctatttggattccgcctgcctggaaagggacttcgcaaaatgatgtggggtatggagcctatgatctttatgatttaggggaatttaatcaaaaggggacggttcgtactaagtatgggacacgtagtcaattggagtctgccatccatgctttaaagaataatggcgttcaagtttatggggatgtagtgatgaaccataaaggaggagctgatgctacagaaaacgttcttgctgtcgaggtgaatccaaataaccggaatcaagaaatatctggggactacacaattgaggcttggactaagtttgattttccagggaggggtaatacatactcagactttaaatggcgttggtatcatttcgatggtgtagattgggatcaatcacgacaattccaaaatcgtatctacaaattccgaggtgatggtaaggcatgggattgggaagtagattcggaaaatggaaattatgattatttaatgtatgcagatgtagatatggatcatccggaggtagtaaatgagcttagaagatggggagaatggtatacaaatacattaaatcttgatggatttaggatcgatgcggtgaagcatattaaatatagctttacacgtgattggttgacccatgtaagaaacgcaacgggaaaagaaatgtttgctgttgctgaattttggaaaaatgatttaggtgccttggagaactatttaaataaaacaaactggaatcattctgtctttgatgtcccccttcattataatctttataacgcgtcaaatagtggaggcaactatgacatggcaaaacttcttaatggaacggttgttcaaaagcatccaatgcatgccgtaacttttgtggataatcacgattctcaacctggggaatcattagaatcatttgtacaagaatggtttaagccacttgcttatgcgcttattttaacaagagaacaaggctatccctctgtcttctatggtgactactatggaattccaacacatagtgtcccagcaatgaaagccaagattgatccaatcttagaggcgcgtcaaaattttgcatatggaacacaacatgattattttgaccatcataatataatcggatggacacgtgaaggaaataccacgcatcccaattcaggacttgcgactatcatgtcggatgggccagggggagagaaatggatgtacgtagggcaaaataaagcaggtcaagtttggcatgacataactggaaataaaccaggaacagttacgatcaatgcagatggatgggctaatttttcagtaaatggaggatctgtttccatttgggtgaaacga

SEQ ID NO: 4 - protein, 485 aa, Bacillus SP722
HHNGTNGTMMQYFEWHLPNDGNHWNRLRDDASNLRNRGITAIWIPPAWKGTSQNDVGYGAYDLYDLGEFNQKGTVRTKYGTRSQLESAIHALKNNGVQVYGDVVMNHKGGADATENVLAVEVNPNNRNQEISGDYTIEAWTKFDFPGRGNTYSDFKWRWYHFDGVDWDQSRQFQNRIYKFRGDGKAWDWEVDSENGNYDYLMYADVDMDHPEVVNELRRWGEWYTNTLNLDGFRIDAVKHIKYSFTRDWLTHVRNATGKEMFAVAEFWKNDLGALENYLNKTNWNHSVFDVPLHYNLYNASNSGGNYDMAKLLNGTVVQKHPMHAVTFVDNHDSQPGESLESFVQEWFKPLAYALILTREQGYPSVFYGDYYGIPTHSVPAMKAKIDPILEARQNFAYGTQHDYFDHHNIIGWTREGNTTHPNSGLATIMSDGPGGEKWMYVGQNKAGQVWHDITGNKPGTVTINADGWANFSVNGGSVSIWVKR

SEQ ID NO: 5 - DNA, 1548 bp, Bacillus BSG
  source 1..1548: mol_type = genomic DNA
  CDS 1..1548
gccgcaccgtttaacggcaccatgatgcagtattttgaatggtacttgccggatgatggcacgttatggaccaaagtggccaatgaagccaacaacttatccagccttggcatcaccgctctttggctgccgcccgcttacaaaggaacaagccgcagcgacgtagggtacggagtatacgacttgtatgacctcggcgaattcaatcaaaaagggaccgtccgcacaaaatacggaacaaaagctcaatatcttcaagccattcaagccgcccacgccgctggaatgcaagtgtacgccgatgtcgtgttcgaccataaaggcggcgctgacggcacggaatgggtggacgccgtcgaagtcaatccgtccgaccgcaaccaagaaatctcgggcacctatcaaatccaagcatggacgaaatttgattttcccgggcggggcaacacctactccagctttaagtggcgctggtaccattttgacggcgttgattgggacgaaagccgaaaattgagccgcatttacaaattccgcggcatcggcaaagcgtgggattgggaagtagacacggaaaacggaaactatgactacttaatgtatgccgaccttgatatggatcatcccgaagtcgtgaccgagctgaaaaactgggggaaatggtatgtcaacacaacgaacattgatgggttccggcttgatgccgtcaagcatattaagttcagtttttttcctgattggttgtcgtatgtgcgttctcagactggcaagccgctatttaccgtcggggaatattggagctatgacatcaacaagttgcacaattacattacgaaaacagacggaacgatgtctttgtttgatgccccgttacacaacaaattttataccgcttccaaatcagggggcgcatttgatatgcgcacgttaatgaccaatactctcatgaaagatcaaccgacattggccgtcaccttcgttgataatcatgacaccgaacccggccaagcgctgcagtcatgggtcgacccatggttcaaaccgttggcttacgcctttattctaactcggcaggaaggatacccgtgcgtcttttatggtgactattatggcattccacaatataacattccttcgctgaaaagcaaaatcgatccgctcctcatcgcgcgcagggattatgcttacggaacgcaacatgattatcttgatcactccgacatcatcgggtggacaagggaagggggcactgaaaaaccaggatccggactggccgcactgatcaccgatgggccgggaggaagcaaatggatgtacgttggcaaacaacacgctggaaaagtgttctatgaccttaccggcaaccggagtgacaccgtcaccatcaacagtgatggatggggggaattcaaagtcaatggcggttcggtttcggtttgggttcctagaaaaacgaccgtttctaccatcgctcggccgatcacaacccgaccgtggactggtgaattcgtccgttggaccgaaccacggttggtggcatggccttga

SEQ ID NO: 6 - protein, 515 aa, Bacillus BSG
AAPFNGTMMQYFEWYLPDDGTLWTKVANEANNLSSLGITALWLPPAYKGTSRSDVGYGVYDLYDLGEFNQKGTVRTKYGTKAQYLQAIQAAHAAGMQVYADVVFDHKGGADGTEWVDAVEVNPSDRNQEISGTYQIQAWTKFDFPGRGNTYSSFKWRWYHFDGVDWDESRKLSRIYKFRGIGKAWDWEVDTENGNYDYLMYADLDMDHPEVVTELKNWGKWYVNTTNIDGFRLDAVKHIKFSFFPDWLSYVRSQTGKPLFTVGEYWSYDINKLHNYITKTDGTMSLFDAPLHNKFYTASKSGGAFDMRTLMTNTLMKDQPTLAVTFVDNHDTEPGQALQSWVDPWFKPLAYAFILTRQEGYPCVFYGDYYGIPQYNIPSLKSKIDPLLIARRDYAYGTQHDYLDHSDIIGWTREGGTEKPGSGLAALITDGPGGSKWMYVGKQHAGKVFYDLTGNRSDTVTINSDGWGEFKVNGGSVSVWVPRKTTVSTIARPITTRPWTGEFVRWTEPRLVAWP

SEQ ID NO: 7 - DNA, 1920 bp, Bacillus licheniformis
  source 1..1920: mol_type = genomic DNA
  CDS 421..1872
cggaagattggaagtacaaaaataagcaaaagattgtcaatcatgtcatgagccatgcgggagacggaaaaatcgtcttaatgcacgatatttatgcaacgttcgcagatgctgctgaagagattattaaaaagctgaaagcaaaaggctatcaattggtaactgtatctcagcttgaagaagtgaagaagcagagaggctattgaataaatgagtagaagcgccatatcggcgcttttcttttggaagaaaatatagggaaaatggtacttgttaaaaattcggaatatttatacaacatcatatgtttcacattgaaaggggaggagaatcatgaaacaacaaaaacggctttacgcccgattgctgacgctgttatttgcgctcatcttcttgctgcctcattctgcagcagcggcggcaaatcttaatgggacgctgatgcagtattttgaatggtacatgcccaatgacggccaacattggaggcgtttgcaaaacgactcggcatatttggctgaacacggtattactgccgtctggattcccccggcatataagggaacgagccaagcggatgtgggctacggtgcttacgacctttatgatttaggggagtttcatcaaaaagggacggttcggacaaagtacggcacaaaaggagagctgcaatctgcgatcaaaagtcttcattcccgcgacattaacgtttacggggatgtggtcatcaaccacaaaggcggcgctgatgcgaccgaagatgtaaccgcggttgaagtcgatcccgctgaccgcaaccgcgtaatttcaggagaacacctaattaaagcctggacacattttcattttccggggcgcggcagcacatacagcgattttaaatggcattggtaccattttgacggaaccgattgggacgagtcccgaaagctgaaccgcatctataagtttcaaggaaaggcttgggattgggaagtttccaatgaaaacggcaactatgattatttgatgtatgccgacatcgattatgaccatcctgatgtcgcagcagaaattaagagatggggcacttggtatgccaatgaactgcaattggacggtttccgtcttgatgctgtcaaacacattaaattttcttttttgcgggattgggttaatcatgtcagggaaaaaacggggaaggaaatgtttacggtagctgaatattggcagaatgacttgggcgcgctggaaaactatttgaacaaaacaaattttaatcattcagtgtttgacgtgccgcttcattatcagttccatgctgcatcgacacagggaggcggctatgatatgaggaaattgctgaacggtacggtcgtttccaagcatccgttgaaatcggttacatttgtcgataaccatgatacacagccggggcaatcgcttgagtcgactgtccaaacatggtttaagccgcttgcttacgcttttattctcacaagggaatctggataccctcaggttttctacggggatatgtacgggacgaaaggagactcccagcgcgaaattcctgccttgaaacacaaaattgaaccgatcttaaaagcgagaaaacagtatgcgtacggagcacagcatgattatttcgaccaccatgacattgtcggctggacaagggaaggcgacagctcggttgcaaattcaggtttggcggcattaataacagacggacccggtggggcaaagcgaatgtatgtcggccggcaaaacgccggtgagacatggcatgacattaccggaaaccgttcggagccggttgtcatcaattcggaaggctggggagagtttcacgtaaacggcgggtcggtttcaatttatgttcaaagatagaagagcagagaggacggatttcctgaaggaaatccgtttttttatttt

SEQ ID NO: 8 - protein, 483 aa, Bacillus licheniformis [sequence omitted]

SEQ ID NO: 9 - DNA, 2084 bp, Bacillus BAN
  source 1..2084: mol_type = genomic DNA
  CDS 343..1794
gccccgcacatacgaaaagactggctgaaaacattgagcctttgatgactgatgatttggctgaagaagtggatcgattgtttgagaaaagaagaagaccataaaaataccttgtctgtcatcagacagggtattttttatgctgtccagactgtccgctgtgtaaaaataaggaataaaggggggttgttattattttactgatatgtaaaatataatttgtataagaaaatgagagggagaggaaacatgattcaaaaacgaaagcggacagtttcgttcagacttgtgcttatgtgcacgctgttatttgtcagtttgccgattacaaaaacatcagccgtaaatggcacgctgatgcagtattttgaatggtatacgccgaacgacggccagcattggaaacgattgcagaatgatgcggaacatttatcggatatcggaatcactgccgtctggattcctcccgcatacaaaggattgagccaatccgataacggatacggaccttatgatttgtatgatttaggagaattccagcaaaaagggacggtcagaacgaaatacggcacaaaatcagagcttcaagatgcgatcggctcactgcattcccggaacgtccaagtatacggagatgtggttttgaatcataaggctggtgctgatgcaacagaagatgtaactgccgtcgaagtcaatccggccaatagaaatcaggaaacttcggaggaatatcaaatcaaagcgtggacggattttcgttttccgggccgtggaaacacgtacagtgattttaaatggcattggtatcatttcgacggagcggactgggatgaatcccggaagatcagccgcatctttaagtttcgtggggaaggaaaagcgtgggattgggaagtatcaagtgaaaacggcaactatgactatttaatgtatgctgatgttgactacgaccaccctgatgtcgtggcagagacaaaaaaatggggtatctggtatgcgaatgaactgtcattagacggcttccgtattgatgccgccaaacatattaaattttcatttctgcgtgattgggttcaggcggtcagacaggcgacgggaaaagaaatgtttacggttgcggagtattggcagaataatgccgggaaactcgaaaactacttgaataaaacaagctttaatcaatccgtgtttgatgttccgcttcatttcaatttacaggcggcttcctcacaaggaggcggatatgatatgaggcgtttgctggacggtaccgttgtgtccaggcatccggaaaaggcggttacatttgttgaaaatcatgacacacagccgggacagtcattggaatcgacagtccaaacttggtttaaaccgcttgcatacgcctttattttgacaagagaatccggttatcctcaggtgttctatggggatatgtacgggacaaaagggacatcgccaaaggaaattccctcactgaaagataatatagagccgattttaaaagcgcgtaaggagtacgcatacgggccccagcacgattatattgaccacccggatgtgatcggatggacgagggaaggtgacagctccgccgccaaatcaggtttggccgctttaatcacggacggacccggcggatcaaagcggatgtatgccggcctgaaaaatgccggcgagacatggtatgacataacgggcaaccgttcagatactgtaaaaatcggatctgacggctggggagagtttcatgtaaacgatgggtccgtctccatttatgttcagaaataaggtaataaaaaaacacctccaagctgagtgcgggtatcagcttggaggtgcgtttattttttcagccgtatgacaaggtcggcatcaggtgtgacaaatacggtatgctggctgtcataggtgacaaatccgggttttgcgccgtttggctttttcacatgtctgatttttgtataatcaacaggcacggagccggaatctttcgccttggaaaaataagcggcgatcgtagctgcttccaatatggattgttcatcgggatcgctgcttttaatcacaacgtgggatcc

SEQ ID NO: 10 - protein, 483 aa, Bacillus BAN
VNGTLMQYFEWYTPNDGQHWKRLQNDAEHLSDIGITAVWIPPAYKGLSQSDNGYGPYDLYDLGEFQQKGTVRTKYGTKSELQDAIGSLHSRNVQVYGDVVLNHKAGADATEDVTAVEVNPANRNQETSEEYQIKAWTDFRFPGRGNTYSDFKWHWYHFDGADWDESRKISRIFKFRGEGKAWDWEVSSENGNYDYLMYADVDYDHPDVVAETKKWGIWYANELSLDGFRIDAAKHIKFSFLRDWVQAVRQATGKEMFTVAEYWQNNAGKLENYLNKTSFNQSVFDVPLHFNLQAASSQGGGYDMRRLLDGTVVSRHPEKAVTFVENHDTQPGQSLESTVQTWFKPLAYAFILTRESGYPQVFYGDMYGTKGTSPKEIPSLKDNIEPILKARKEYAYGPQHDYIDHPDVIGWTREGDSSAAKSGLAALITDGPGGSKRMYAGLKNAGETWYDITGNRSDTVKIGSDGWGEFHVNDGSVSIYVQK

SEQ ID NO: 11 - DNA, 1458 bp, Bacillus AA560
  source 1..1458: mol_type = genomic DNA
caccataatggtacgaacggcacaatgatgcagtactttgaatggtatctaccaaatgacggaaaccattggaatagattaaggtctgatgcaagtaacctaaaagataaagggatctcagcggtttggattcctcctgcatggaagggtgcctctcaaaatgatgtggggtatggtgcttatgatctgtatgatttaggagaattcaatcaaaaaggaaccattcgtacaaaatatggaacgcgcaatcagttacaagctgcagttaacgccttgaaaagtaatggaattcaagtgtatggcgatgttgtaatgaatcataaagggggagcagacgctaccgaaatggttagggcagttgaagtaaacccgaataatagaaatcaagaagtgtccggtgaatatacaattgaggcttggacaaagtttgactttccaggacgaggtaatactcattcaaacttcaaatggagatggtatcactttgatggagtagattgggatcagtcacgtaagctgaacaatcgaatttataaatttagaggtgatggaaaagggtgggattgggaagtcgatacagaaaacggtaactatgattacctaatgtatgcagatattgacatggatcacccagaggtagtgaatgagctaagaaattggggtgtttggtatacgaatacattaggccttgatggttttagaatagatgcagtaaaacatataaaatacagctttactcgtgattggattaatcatgttagaagtgcaactggcaaaaatatgtttgcggttgcggaattttggaaaaatgatttaggtgctattgaaaactatttaaacaaaacaaactggaaccattcagtctttgatgttccgctgcactataacctctataatgcttcaaaaagcggagggaattatgatatgaggcaaatatttaatggtacagtcgtgcaaagacatccaatgcatgctgttacatttgttgataatcatgattcgcaacctgaagaagctttagagtcttttgttgaagaatggttcaaaccattagcgtatgctttgacattaacacgtgaacaaggctacccttctgtattttatggagattattatggcattccaacgcatggtgtaccagcgatgaaatcgaaaattgacccgattctagaagcgcgtcaaaagtatgcatatggaagacaaaatgactacttagaccatcataatatcatcggttggacacgtgaagggaatacagcacaccccaactccggtttagctactatcatgtccgatggggcaggaggaaataagtggatgtttgttgggcgtaataaagctggtcaagtttggaccgatatcactggaaatcgtgcaggtactgttacgattaatgctgatggatggggtaatttttctgtaaatggaggatcagtttctatttgggtaaacaaataa

SEQ ID NO: 12 - protein, 485 aa, Bacillus AA560
HHNGTNGTMMQYFEWYLPNDGNHWNRLRSDASNLKDKGISAVWIPPAWKGASQNDVGYGAYDLYDLGEFNQKGTIRTKYGTRNQLQAAVNALKSNGIQVYGDVVMNHKGGADATEMVRAVEVNPNNRNQEVSGEYTIEAWTKFDFPGRGNTHSNFKWRWYHFDGVDWDQSRKLNNRIYKFRGDGKGWDWEVDTENGNYDYLMYADIDMDHPEVVNELRNWGVWYTNTLGLDGFRIDAVKHIKYSFTRDWINHVRSATGKNMFAVAEFWKNDLGAIENYLNKTNWNHSVFDVPLHYNLYNASKSGGNYDMRQIFNGTVVQRHPMHAVTFVDNHDSQPEEALESFVEEWFKPLAYALTLTREQGYPSVFYGDYYGIPTHGVPAMKSKIDPILEARQKYAYGRQNDYLDHHNIIGWTREGNTAHPNSGLATIMSDGAGGNKWMFVGRNKAGQVWTDITGNRAGTVTINADGWGNFSVNGGSVSIWVNK

SEQ ID NO: 13 - protein, 586 aa, Bacillus AMY1048
GSVPVNGTMMQYFEWYLPDDGTLWTKVANNAQSLANLGITALWLPPAYKGTSSSDVGYGVYDLYDLGEFNQKGTVRTKYGTKTQYIQAIQAAHTAGMQVYADVVFNHKAGADGTELVDAVEVNPSDRNQEISGTYQIQAWTKFDFPGRGNTYSSFKWRWYHFDGTDWDESRKLNRIYKFRGTGKAWDWEVDTENGNYDYLMYADLDMDHPEVVSELKNWGKWYVTTTNIDGFRLDAVKHIKYSFFPDWLSYVRTQTQKPLFAVGEFWSYDISKLHNYITKTNGSMSLFDAPLHNNFYIASKSGGYFDMRTLLNNTLMKDQPTLAVTLVDNHDTEPGQSLQSWVEPWFKPLAYAFILTRQEGYPCVFYGDYYGIPKYNIPALKSKLDPLLIARRDYAYGTQHDYIDSADIIGWTREGVAEKANSGLAALITDGPGGSKWMYVGKQHAGKTFYDLTGNRSDTVTINADGWGEFKVNGGSVSIWVPKISTTSQITFTVNNATTVWGQNVYVVGNISQLGNWDPVHAVQMTPSSYPTWTVTIPLLQGQNIQFKFIKKDSAGNVIWEDISNRTYTVPTAASGAYTASWNVP

SEQ ID NO: 14 - protein, 486 aa, Bacillus AMRK385
HHNGTNGTMMQYFEWHLPNDGQHWNRLRNDAANLKNLGITAVWIPPAWKGTSQNDVGYGAYDLYDLGEFNQKGTIRTKYGTRSQLQSAIASLQNNGIQVYGDVVMNHKGGADGTEWVQAVEVNPSNRNQEVTGEYTIEAWTKFDFPGRGNTHSSFKWRWYHFDGTDWDQSRQLNNRIYKFRGTGKAWDWEVDTENGNYDYLMYADVDMDHPEVINELRRWGVWYTNTLNLDGFRIDAVKHIKYSFTRDWLNHVRSTTGKNNMFAVAEFWKNDLGAIENYLHKTNWNHSVFDVPLHYNLYNASKSGGNYDMRQILNGTVVSKHPIHAVTFVDNHDSQPGEALESFVEAWFKPLAYALILTREQGYPSVFYGDYYGIPTHGVAAMKGKIDPILEARQKYAYGTQHDYLDHHNIIGWTREGNSAHPNSGLATIMSDGPGGSKWMYVGRHKAGQVWRDITGNRTGTVTINADGWGNFSVNGGSVSIWVNK

SEQ ID NO: 15 - protein, 480 aa, Bacillus SP.K38
DGLNGTMMQYYEWHLENDGQHWNRLHDDAAALSDAGITAIWIPPAYKGNSQADVGYGAYDLYDLGEFNQKGTVRTKYGTKAQLERAIGSLKSNDINVYGDVVMNHKMGADFTEAVQAVQVNPTNRWQDISGAYTIDAWTGFDFSGRNNAYSDFKWRWFHFNGVDWDQRYQENHIFRFANTNWNWRVDEENGNYDYLLGSNIDFSHPEVQDELKDWGSWFTDELDLDGYRLDAIKHIPFWYTSDWVRHQRNEADQDLFVVGEYWKDDVGALEFYLDEMNWEMSLFDVPLNYNFYRASQQGGSYDMRNILRGSLVEAHPMHAVTFVDNHDTQPGESLESWVADWFKPLAYATILTREGGYPNVFYGDYYGIPNDNISAKKDMIDELLDARQNYAYGTQHDYFDHWDVVGWTREGSSSRPNSGLATIMSNGPGGSKWMYVGRQNAGQTWTDLTGNNGASVTINGDGWGEFFTNGGSVSVYVNQ

SEQ ID NO: 16 - protein, 485 aa, Bacillus AAI-10
HHDGTNGTIMQYFEWNVPNDGQHWNRLHNNAQNLKNAGITAIWIPPAWKGTSQNDVGYGAYDLYDLGEFNQKGTVRTKYGTKAELERAIRSLKANGIQVYGDVVMNHKGGADFTERVQAVEVNPQNRNQEVSGTYQIEAWTGFNFPGRGNQHSSFKWRWYHFDGTDWDQSRQLANRIYKFRGDGKAWDWEVDTENGNYDYLMYADVDMDHPEVINELNRWGVWYANTLNLDGFRLDAVKHIKFSFMRDWLGHVRGQTGKNLFAVAEYWKNDLGALENYLSKTNWTMSAFDVPLHYNLYQASNSSGNYDMRNLLNGTLVQRHPSHAVTFVDNHDTQPGEALESFVQGWFKPLAYATILTREQGYPQVFYGDYYGIPSDGVPSYRQQIDPLLKARQQYAYGRQHDYFDHWDVIGWTREGNASHPNSGLATIMSDGPGGSKWMYVGRQKAGEVWHDMTGNRSGTVTINQDGWGHFFVNGGSVSVWVKR

SEQ ID NO: 17 - protein, 485 aa, Bacillus KSM-AP1378
HHNGTNGTMMQYFEWHLPNDGNHWNRLRDDAANLKSKGITAVWIPPAWKGTSQNDVGYGAYDLYDLGEFNQKGTVRTKYGTRSQLQGAVTSLKNNGIQVYGDVVMNHKGGADGTEMVNAVEVNRSNRNQEISGEYTIEAWTKFDFPGRGNTHSNFKWRWYHFDGTDWDQSRQLQNKIYKFRGTGKAWDWEVDIENGNYDYLMYADIDMDHPEVINELRNWGVWYTNTLNLDGFRIDAVKHIKYSYTRDWLTHVRNTTGKPMFAVAEFWKNDLAAIENYLNKTSWNHSVFDVPLHYNLYNASNSGGYRDMRNILNGSVVQKHPIHAVTFVDNHDSQPGEALESFVQSWFKPLAYALILTREQGYPSVFYGDYYGIPTHGVPSMKSKIDPLLQARQTYAYGTQHDYFDHHDIIGWTREGDSSHPNSGLATIMSDGPGGNKWMYVGKHKAGQVWRDITGNRSGTVTINADGWGNFTVNGGAVSVWVKQ

SEQ ID NO: 18 - protein, 485 aa, Bacillus SP.7-7
HHNGTNGTMMQYFEWYLPNDGNHWNRLRSDASNLKDKGITAVWIPPAWKGASQNDVGYGAYDLYDLGEFNQKGTVRTKYGTRNQLQAAVTALKSNGIQVYGDVVMNHKGGADATEWVRAVEVNPSNRNQEVSGDYTIEAWTKFDFPGRGNTHSNFKWRWYHFDGVDWDQSRQLQNRIYKFRGDGKGWDWEVDTENGNYDYLMYADIDMDHPEVVNELRNWGVWYTNTLGLDGFRIGAVKHIKYSFTRDWLTHVRNTTGKNMFAVAEFWKNDIGAIENYLSKTNWNHSVFDVPLHYNLYNASRSGGNYDMRQIFNGTVVQRHPTHAVTFVDNHDSQPEEALESFVEEWFKPLACALTLTRDQGYPSVFYGDYYGIPTHGVPAMKSKIDPILEARQKYAYGKQNDYLDHHNMIGWTREGNTAHPNSGLATIMSDGPGGNKWMYVGRNKAGQVWRDITGNRSGTVTINADGWGNFSVNGGSVSIWVNN